European Patent Specification EP 3 597 737 B1, published September 16, 2026. Title: PROCESS FOR PREPARING BETA 3 AGONISTS AND INTERMEDIATES. Applicant: MERCK SHARP & DOHME CORP. Xu, Feng Liu, Zhuqing Desmond, Richard Park, Jeonghan Kalinin, Alexei Kosjek, Birgit Strotman, Hallena Li, Hongmei Moncecchi, Johannah. Application EP 14 76 8236.3. The sequence listing filed with the application follows.

SEQUENCE LISTING (1 sequence)

SEQ ID NO: 1 - protein, 252 aa, Artificial Sequence
  Engineered variant of Lactobacillus kefir ketoreductase
MTDRLKGKVAIVTGGTQGIGLAIADKFVEEGAKVVITGRRADVGEKAAKSIGGTDVIRFVQHDVSDEAGWPKLFDTTEEAFGPVTTVVNNAGIPMVKSVEDTTTEEWRKLLSVNLDGVFFGARLGIQRMKNKGLGASIINMSSVFGIVGDPTTGAYCASKGAVRIMSKSAALDCALKDYDVRVNTVHPGPIKTPMMDSYEGAEEMFSQRTKTPMGHIGEPNDIAWVCVYLASDESKFATGAEFVVDGGFTAQ